European Patent Specification EP 3 390 669 B1, published July 31, 2024. Title: BIOMARKERS OF CHRONIC LYMPHOCYTIC LEUKEMIA AND USE THEREOF. Applicant: The National Institute for Biotechnology in the Negev Ltd. The sequence listing filed with the application follows.

SEQUENCE LISTING (16 sequences)

SEQ ID NO: 1 - RNA, 23 nt, Artificial sequence
  siRNA
aaguugaucuucagacagcccuu

SEQ ID NO: 2 - RNA, 23 nt, Artificial sequence
  siRNA
aagggcugucugaagaucaacuu

SEQ ID NO: 3 - RNA, 23 nt, Artificial sequence
  siRNA
aauccuggguccaguguggaauu

SEQ ID NO: 4 - RNA, 23 nt, Artificial sequence
  siRNA
aauuccacacuggacccaggauu

SEQ ID NO: 5 - RNA, 25 nt, Artificial sequence
  siRNA
cagagacgguuaucaagagacuaaa

SEQ ID NO: 6 - RNA, 25 nt, Artificial sequence
  siRNA
uuuagucucuugauaaccgucucug

SEQ ID NO: 7 - RNA, 25 nt, Artificial sequence
  siRNA
ccaacaagauuuggcccuauguaua

SEQ ID NO: 8 - RNA, 25 nt, Artificial sequence
  siRNA
uauacauagggccaaaucuuguugg

SEQ ID NO: 9 - RNA, 19 nt, Artificial sequence
  siRNA
gcaaacaucccagagguau

SEQ ID NO: 10 - RNA, 19 nt, Artificial sequence
  siRNA
auaccucugggauguuugc

SEQ ID NO: 11 - DNA, 22 bp, Artificial sequence
  Primer
gccccaaaccaattaaatcctg

SEQ ID NO: 12 - DNA, 22 bp, Artificial sequence
  Primer
caatgccaatcaaatctcgtcc

SEQ ID NO: 13 - DNA, 21 bp, Artificial sequence
  Primer
ttactgctcgctggattcatc

SEQ ID NO: 14 - DNA, 22 bp, Artificial sequence
  Primer
gtctcttgataaccgtctctgg

SEQ ID NO: 15 - DNA, 20 bp, Artificial sequence
  Primer
actcttccagccttccttcc

SEQ ID NO: 16 - DNA, 20 bp, Artificial sequence
  Primer
tgttggcgtacaggtctttg